European Patent Specification EP 3 265 112 B1, published December 24, 2025. Title: UBIQUITIN LIGASE KPC1 PROMOTES PROCESSING OF P105 NF-KAPAB1 TO P50, ELICITING STRONG TUMOR SUPPRESSION. Applicant: RAPPAPORT FAMILY INSTITUTE FOR RESEARCH IN THE MEDICAL SCIENCES CIECHANOVER, Aaron KRAVTSOVA, Yelena SHOMER, Inna COHEN, Victoria. The sequence listing filed with the application follows.

SEQUENCE LISTING (18 sequences)

SEQ ID NO: 1 - protein, 969 aa, Homo sapiens
MAEDDPYLGRPEQMFHLDPSLTHTIFNPEVFQPQMALPTADGPYLQILEQPKQRGFRFRYVCEGPSHGGLPGASSEKNKKSYPQVKICNYVGPAKVIVQLVTNGKNIHLHAHSLVGKHCEDGICTVTAGPKDMVVGFANLGILHVTKKKVFETLEARMTEACIRGYNPGLLVHPDLAYLQAEGGGDRQLGDREKELIRQAALQQTKEMDLSVVRLMFTAFLPDSTGSFTRRLEPVVSDAIYDSKAPNASNLKIVRMDRTAGCVTGGEEIYLLCDKVQKDDIQIRFYEEEENGGVWEGFGDFSPTDVHRQFAIVFKTPKYKDINITKPASVFVQLRRKSDLETSEPKPFLYYPEIKDKEEVQRKRQKLMPNFSDSFGGGSGAGAGGGGMFGSGGGGGGTGSTGPGYSFPHYGFPTYGGITFHPGTTKSNAGMKHGTMDTESKKDPEGCDKSDDKNTVNLFGKVIETTEQDQEPSEATVGNGEVTLTYATGTKEESAGVQDNLFLEKAMQLAKRHANALFDYAVTGDVKMLLAVQRHLTAVQDENGDSVLHLAIIHLHSQLVRDLLEVTSGLISDDIINMRNDLYQTPLHLAVITKQEDVVEDLLRAGADLSLLDRLGNSVLHLAAKEGHDKVLSILLKHKKAALLLDHPNGDGLNAIHLAMMSNSLPCLLLLVAAGADVNAQEQKSGRTALHLAVEHDNISLAGCLLLEGDAHVDSTTYDGTTPLHIAAGRGSTRLAALLKAAGADPLVENFEPLYDLDDSWENAGEDEGVVPGTTPLDMATSWQVFDILNGKPYEPEFTSDDLLAQGDMKQLAEDVKLQLYKLLEIPDPDKNWATLAQKLGLGILNNAFRLSPAPSKTLMDNYEVSGGTVRELVEALRQMGYTEAIEVIQAASSPVKTTSQAHSLPLSPASTRQQIDELRDSDSVCDSGVETSFRKLSFTESLTSGASLLTLNKMPHDYGQEGPLEGKI

SEQ ID NO: 2 - DNA, 2910 bp, Homo sapiens
atggcagaagatgatccatatttgggaaggcctgaacaaatgtttcatttggatccttctttgactcatacaatatttaatccagaagtatttcaaccacagatggcactgccaacagcagatggcccataccttcaaatattagagcaacctaaacagagaggatttcgtttccgttatgtatgtgaaggcccatcccatggtggactacctggtgcctctagtgaaaagaacaagaagtcttaccctcaggtcaaaatctgcaactatgtgggaccagcaaaggttattgttcagttggtcacaaatggaaaaaatatccacctgcatgcccacagcctggtgggaaaacactgtgaggatgggatctgcactgtaactgctggacccaaggacatggtggtcggcttcgcaaacctgggtatacttcatgtgacaaagaaaaaagtatttgaaacactggaagcacgaatgacagaggcgtgtataaggggctataatcctggactcttggtgcaccctgaccttgcctatttgcaagcagaaggtggaggggaccggcagctgggagatcgggaaaaagagctaatccgccaagcagctctgcagcagaccaaggagatggacctcagcgtggtgcggctcatgtttacagcttttcttccggatagcactggcagcttcacaaggcgcctggaacccgtggtatcagacgccatctatgacagtaaagcccccaatgcatccaacttgaaaattgtaagaatggacaggacagctggatgtgtgactggaggggaggaaatttatcttctttgtgacaaagttcagaaagatgacatccagattcgattttatgaagaggaagaaaatggtggagtctgggaaggatttggagatttttcccccacagatgttcatagacaatttgccattgtcttcaaaactccaaagtataaagatattaatattacaaaaccagcctctgtgtttgtccagcttcggaggaaatctgacttggaaactagtgaaccaaaacctttcctctactatcctgaaatcaaagataaagaagaagtgcagaggaaacgtcagaagctcatgcccaatttttcggatagtttcggcggtggtagtggtgctggagctggaggcggaggcatgtttggtagtggcggtggaggagggggcactggaagtacaggtccagggtatagcttcccacactatggatttcctacttatggtgggattactttccatcctggaactactaaatctaatgctgggatgaagcatggaaccatggacactgaatctaaaaaggaccctgaaggttgtgacaaaagtgatgacaaaaacactgtaaacctctttgggaaagttattgaaaccacagagcaagatcaggagcccagcgaggccaccgttgggaatggtgaggtcactctaacgtatgcaacaggaacaaaagaagagagtgctggagttcaggataacctctttctagagaaggctatgcagcttgcaaagaggcatgccaatgcccttttcgactacgcggtgacaggagacgtgaagatgctgctggccgtccagcgccatctcactgctgtgcaggatgagaatggggacagtgtcttacacttagcaatcatccaccttcattctcaacttgtgagggatctactagaagtcacatctggtttgatttctgatgacattatcaacatgagaaatgatctgtaccagacgcccttgcacttggcagtgatcactaagcaggaagatgtggtggaggatttgctgagggctggggccgacctgagccttctggaccgcttgggtaactctgttttgcacctagctgccaaagaaggacatgataaagttctcagtatcttactcaagcacaaaaaggcagcactacttcttgaccaccccaacggggacggtctgaatgccattcatctagccatgatgagcaatagcctgccatgtttgctgctgctggtggccgctggggctgacgtcaatgctcaggagcagaagtccgggcgcacagcactgcacctggctgtggagcacgacaacatctcattggcaggctgcctgctcctggagggtgatgcccatgtggacagtactacctacgatggaaccacacccctgcatatagcagctgggagagggtccaccaggctggcagctcttctcaaagcagcaggagcagatcccctggtggagaactttgagcctctctatgacctggatgactcttgggaaaatgcaggagaggatgaaggagttgtgcctggaaccacgcctctagatatggccaccagctggcaggtatttgacatattaaatgggaaaccatatgagccagagtttacatctgatgatttactagcacaaggagacatgaaacagctggctgaagatgtgaagctgcagctgtataagttactagaaattcctgatccagacaaaaactgggctactctggcgcagaaattaggtctggggatacttaataatgccttccggctgagtcctgctccttccaaaacacttatggacaactatgaggtctctgggggtacagtcagagagctggtggaggccctgagacaaatgggctacaccgaagcaattgaagtgatccaggcagcctccagcccagtgaagaccacctctcaggcccactcgctgcctctctcgcctgcctccacaaggcagcaaatagacgagctccgagacagtgacagtgtctgcgacagcggcgtggagacatccttccgcaaactcagctttaccgagtctctgaccagtggtgcctcactgctaactctcaacaaaatgccccatgattatgggcaggaaggacctctagaaggcaaaatttag

SEQ ID NO: 3 - protein, 434 aa, Homo sapiens
MAEDDPYLGRPEQMFHLDPSLTHTIFNPEVFQPQMALPTADGPYLQILEQPKQRGFRFRYVCEGPSHGGLPGASSEKNKKSYPQVKICNYVGPAKVIVQLVTNGKNIHLHAHSLVGKHCEDGICTVTAGPKDMVVGFANLGILHVTKKKVFETLEARMTEACIRGYNPGLLVHPDLAYLQAEGGGDRQLGDREKELIRQAALQQTKEMDLSVVRLMFTAFLPDSTGSFTRRLEPVVSDAIYDSKAPNASNLKIVRMDRTAGCVTGGEEIYLLCDKVQKDDIQIRFYEEEENGGVWEGFGDFSPTDVHRQFAIVFKTPKYKDINITKPASVFVQLRRKSDLETSEPKPFLYYPEIKDKEEVQRKRQKLPNFSDSFGGGSGAGAGGGGMFGSGGGGGGTGSTGPGYSFPHYGFPTYGGITFHPGTTKSNAGMKHGT

SEQ ID NO: 4 - protein, 1314 aa, Homo sapiens
MASKGAGMSFSRKSYRLTSDAEKSRVTGIVQEKLLNDYLNRIFSSSEHAPPAATSRKPLNFQNLPEHLDQLLQVDNEEEESQGQVEGRLGPSTVVLDHTGGFEGLLLVDDDLLGVIGHSNFGTIRSTTCVYKGKWLYEVLISSQGLMQIGWCTISCRFNQEEGVGDTHNSYAYDGNRVRKWNVTTTNYGKAWAAGDIVSCLIDLDDGTLSFCLNGVSLGTAFENLSRGLGMAYFPAISLSFKESVAFNFGSRPLRYPVAGYRPLQDPPSADLVRAQRLLGCFRAVLSVELDPVEGRLLDKESSKWRLRGQPTVLLTLAHIFHHFAPLLRKVYLVEAVLMSFLLGIVEKGTPTQAQSVVHQVLDLLWLFMEDYEVQDCLKQLMMSLLRLYRFSPIVPDLGLQIHYLRLTIAILRHEKSRKFLLSNVLFDVLRSVVFFYIKSPLRVEEAGLQELIPTTWWPHCSSREGKESTEMKEETAEERLRRRAYERGCQRLRKRIEVVEELQVQILKLLLDNKDDNGGEASRYIFLTKFRKFLQENASGRGNMPMLCPPEYMVCFLHRLISALRYYWDEYKASNPHASFSEEAYIPPQVFYNGKVDYFDLQRLGGLLSHLRKTLKDDLASKANIVIDPLELQSTAMDDLDEDEEPAPAMAQRPMQALAVGGPLPLPRPGWLSSPTLGRANRFLSTAAVSLMTPRRPLSTSEKVKVRTLSVEQRTREDIEGSHWNEGLLLGRPPEEPEQPLTENSLLEVLDGAVMMYNLSVHQQLGKMVGVSDDVNEYAMALRDTEDKLRRCPKRRKDILAELTKSQKVFSEKLDHLSRRLAWVHATVYSQEKMLDIYWLLRVCLRTIEHGDRTGSLFAFMPEFYLSVAINSYSALKNYFGPVHSMEELPGYEETLTRLAAILAKHFADARIVGTDIRDSLMQALASYVCYPHSLRAVERIPEEQRIAMVRNLLAPYEQRPWAQTNWILVRLWRGCGFGYRYTRLPHLLKTKLEDANLPSLQKPCPSTLLQQHMADLLQQGPDVAPSFLNSVLNQLNWAFSEFIGMIQEIQQAAERLERNFVDSRQLKVCATCFDLSVSLLRVLEMTITLVPEIFLDWTRPTSEMLLRRLAQLLNQVLNRVTAERNLFDRVVTLRLPGLESVDHYPILVAVTGILVQLLVRGPASEREQATSVLLADPCFQLRSICYLLGQPEPPAPGTALPAPDRKRFSLQSYADYISADELAQVEQMLAHLTSASAQAAAASLPTSEEDLCPICYAHPISAVFQPCGHKSCKACINQHLMNNKDCFFCKTTIVSVEDWEKGANTSTTSSAA

SEQ ID NO: 5 - DNA, 3945 bp, Homo sapiens
atggcatccaagggggccggcatgtctttctcccgcaagagctataggctgacctcagatgctgagaaatccagggtcacaggcattgtgcaggagaagctgctgaatgactacctgaaccgcatcttttcctcttctgaacatgcacccccagcagccaccagcaggaaacccctgaacttccagaacctgccagaacatttggaccagttgctacaggtggacaatgaggaggaggaaagccagggacaggttgaagggcggcttggcccatccactgtggtcctggaccacacaggcggctttgaggggcttctcctggtggatgatgacctgctgggggtgattggacacagcaactttggcaccatccgctctaccacatgcgtgtacaaagggaaatggctctacgaggtcctcatctcctcccaggggctcatgcagatcggctggtgcaccatcagctgccgcttcaaccaggaggagggggttggagatacacacaactcctatgcctatgatggcaaccgcgtgcgcaagtggaatgtgaccacaacgaattatggcaaggcgtgggcagcgggggacatcgtgagctgcctgattgacctggatgatggcactctgtccttctgcctgaacggtgtatcactgggcactgcctttgagaacctgtccaggggcctgggtatggcctacttcccagccatcagcctctctttcaaggagtccgtggccttcaactttggcagccgtcctctgcgctacccagtggcaggctaccggcccctgcaggacccaccgagtgctgacctggtgcgggcacagaggttgctgggctgcttccgggcagtgctgagtgtggagctggaccctgtggaggggcggctgttggacaaggagagctccaagtggcggttgcggggccagcccaccgtcctcctcacactggcccacatcttccatcactttgcaccgcttctgcgcaaggtgtatctggtggaggctgtgctcatgagcttcttgctgggcatcgtggagaagggcacacccacacaggcacagtccgtggtgcaccaggtcctggacctcttgtggctcttcatggaggactacgaggtacaagattgcctcaagcagttgatgatgtctctgcttcggctgtaccgattctcacccattgtcccagacctgggcctacagatccattacctgcggctcactatcgccatcctgaggcatgagaagtcccgcaagtttctgcttagcaatgtcctcttcgacgtgctccgctccgtcgtcttcttttacatcaagagccccctgcgtgtggaggaggccggcctgcaggagctcattcccaccacctggtggccccactgctccagtagggagggcaaagagagcacggagatgaaggaggagaccgcagaggagcggctgcggcggcgagcctacgaacggggctgtcagcggctcaggaagcgcatcgaagtggtggaagaactacaggtccagatcctgaagctgctgctggacaataaagatgacaatgggggtgaagcttctaggtatatcttcctgaccaagtttcgcaagtttctgcaggagaacgccagtggccgggggaacatgcccatgctctgcccccctgagtacatggtctgcttcttacaccggctgatctctgccctgcgctactattgggatgaatacaaggcttccaatcctcatgcttccttcagtgaggaggcctacatcccgccccaggtcttctataatggcaaggtggactactttgacctgcagcgcctggggggcctcctctcgcacctgcggaagaccctcaaagatgaccttgcttccaaagccaacattgtgatcgacccactggagctccagtcaaccgccatggatgacctagatgaggatgaggagccagccccagctatggcccagcgccccatgcaggccctggctgttggggggccactgcccctgccccggcccggctggctcagttctccaactttgggccgagccaaccgcttcctcagcacagcggctgtgagcctcatgaccccacggcggcctctgagcacctcggagaaagtgaaggtccgcacgctgagcgtggagcagaggacccgtgaggacattgaaggcagccactggaatgagggcttgctgctggggcggccccccgaggagcctgagcagcccctcaccgagaactcgctgctggaagtcctggatggggcggtcatgatgtacaacctcagcgtacaccagcagctgggcaagatggtgggtgtctccgatgatgtcaatgaatacgctatggctctgagggacacagaggacaagctccgccggtgccccaagaggaggaaggacatccttgcagagttgaccaagagccagaaggttttctcagaaaagctggaccacctgagccgccgtcttgcctgggtccatgccactgtctactcccaggagaagatgctggacatctactggctgctgcgcgtctgcctgcggaccattgagcacggtgatcgcacagggtctctctttgccttcatgcccgagttctacctgagcgtggccatcaacagctacagtgctctcaagaattactttggtcccgtgcacagcatggaggagctcccaggctatgaagagaccctgacccgcctggctgccattctcgccaaacactttgccgacgcacgcattgtgggcactgacatccgagactcactgatgcaggccctggccagctacgtgtgctacccacactccctgcgggctgtggagcgaatccccgaggagcagcgtatcgccatggtgaggaacctcctggcgccctatgagcagcggccctgggcccagaccaactggatcctggtgcggctctggaggggctgtggcttcgggtaccgctatacacggctgccacatctgctgaaaaccaaacttgaggacgccaatttgcccagcctccagaagccctgcccttccaccctgctgcagcagcacatggcggacctcctacagcagggtcctgatgtggcacccagcttcctcaacagcgtcctcaatcagctcaactgggccttctctgaattcattggcatgatccaagagatccagcaggctgctgagcgcctggagcggaactttgtggacagccggcagctcaaggtatgtgccacctgctttgacctctcggtcagcctgctgcgtgtcttggagatgactatcacactggtgcctgagatattccttgactggacccggcctacctctgagatgctgctgcggcgtcttgcacagctgctaaaccaggtgctgaaccgggtgacagctgagaggaacctgtttgatcgtgtggtcaccctacggctgcctggcctagagagcgtggaccactatcccattctggtggcagtgacgggcatcctggtgcagctcctggtgcgtggcccagcctcagagagagagcaagccacatcagtgctcctggcagatccctgcttccagctacgctcaatatgctatctcctgggacagccagagcccccagcacctggcactgctctgccagcccctgaccggaagcgcttctccctgcagagctatgcggattatatcagtgccgatgagctggcccaagtggaacagatgctggcgcacctgacctctgcatctgcccaggcagcagctgcctccctgcccaccagtgaggaggacctctgccccatctgctatgcccaccccatctctgctgtgttccagccctgtggccacaagtcctgcaaagcctgtatcaaccagcacctgatgaacaacaaggactgcttcttctgcaaaaccaccatcgtgtctgtagaggactgggagaagggagccaatacgagtactacctcctcagctgcctag

SEQ ID NO: 6 - protein, 1320 aa, Mus musculus
MASKGTGMSFSRKSYRLTSDAEKSRVTGIVQEKLLSDYLYRIFSPPDRGPAAATSRKPLNFHNLPEHVDQLLQVDSEDNESQGQVEGRLGPSTVVLDHTGGFEGLLLVDDDLLGVIGHSNFGTIRSTTCVYKGKWVYEVLISSQGLMQIGWCTINCRFNQEEGVGDTHNSYAYDGNRVRKWNVTTTNYGKAWAAGDIVSCLIDLDDGTLSFCLNGVSLGTAFENLSRGLGMAYFPAISLSFKESVAFNFGSRPLRYPVAGFRPLQDPPFADLVRAQRLLGCFQAVLSVELDPVEGRLVETESSEWQLQGQPTVLLTLAHIFHHFAPLLRKVYLVEAVLMSFLLGVVEKGTPEQAQSVVHQILDLLWLFMEDYEVQDCLKQLMMSLLRLYRFSPIVPDLGLQIHYLRLTMSILRHEKSRKFLLSNVLFDMLRSVVFFYIKSPLRVEEAGLKELIPTTWWPHRSSRESRDGKEAREETTEERQRRRAYERGCQRLKKRIEVVEELQVQILKLLLDNKDDNGGEASRYIFLTKFRKFLQENASGRGNTPVLCPPEYMVCFLHRLVSALRFYWDEYKASNPRASFSEEAYIPPQIFYNGKVDYFDLQRLGGLLSHLRKTLKDDLASKANIVIDPLELQAATMDDLDEDEEPAPSAAQVWQEGQRPMQALAIGGALPLPRPGWLSSPTLGRANRFLSTAAVSLMTPRRLLSTMEKVKVRSLNVEQRTREDIEGSHWNEGLLLGRPPEEPEQPLTENSLLEVLDGTVMMYNLSVHQQLGKMVGVSDDVNEYAMALRDTEDKLRRCPKRRKDILAELTKSQKVFSEKLDHLSRRLAWVHATVYSQEKMLDIYWLLRVCLRTIEHGDRTGSLFAFMPEFYLSVAINSYSALKNYFGPVHSMEELPGYEETLTRLAAILAKHFADPRIVGTDIRDSLMQALASYVCYPHSLRAVERIPEEQRIAMVRNLLAPYEQRPWAQTNWILVRLWRGCGFGYRYTRLPHLLKTKPEDANLPSLQKPCPSTLLQQHMADLLRQGSDVAPSFLNSVLNQLNWAFSEFIGMIQEIQQAAERLERNFVDSRQLKVCATCFDLSVSLLRVLEMTITLVPEIFLDWSRPTSEMLLRRLAQLLNQVLNRVTAERNLFDRVVTLRLPGLESVDHYPILVAVTGILVRLLVHGPTSETEQATSVLLADPCFQLRSICYLLGQPEPLAPGTTLPAPDRKRFSLQSYTDYISAEELAQVEQMLAHLTAASAQAAAASLPTNEEDLCPICYAHPISAVFQPCGHKSCKACINQHLMNNKDCFFCKATIVSVEDWDKAANTSAMSSAA

SEQ ID NO: 7 - DNA, 3945 bp, Mus musculus
atggcgtccaaggggactggcatgtcgttctcccgaaagagctataggctgacctcagatgctgagaagtccagggtcacaggcatcgtgcaagagaaactactgagcgactatctgtaccgcatcttttcccctcctgaccgtggacccgccgcagccaccagcaggaaaccgctaaacttccataacctgcctgagcacgtggaccagctgctacaggtggacagtgaagacaacgagagccagggacaagttgaaggtcgacttggcccatctactgtggtcctagaccacacaggaggctttgaggggcttctccttgtggatgatgacctcctgggggtgattggacacagcaactttggcactatccgttctaccacatgtgtgtacaaagggaagtgggtctacgaggtgctcatctcctcccagggcctcatgcagatcggctggtgcaccatcaactgccgctttaatcaggaggaaggggttggagacacacataactcctatgcctatgacggcaaccgagtgcgcaagtggaatgttaccaccacgaattatggcaaggcgtgggctgcgggggacattgtcagctgcctaattgatctggatgatgggactctgtccttctgcctgaatggcgtgtcactgggcactgccttcgagaacctttccaggggcctaggaatggcgtacttcccagccatcagcctgtcattcaaggagtctgtggcattcaactttggcagccgtcctttgcgctacccagttgcgggcttccggcccctgcaggaccctccgtttgctgacctggtccgggcacagaggttgctgggctgcttccaggcagtgctaagtgtggagctggaccctgtggaagggcggctggtggagacggagagctctgagtggcagctgcaagggcagcccactgtcctcctcacgctggcccacatcttccatcactttgcaccactgctgcgcaaggtatacctggtggaggctgtgctaatgagcttcctgctgggcgttgtggagaagggcacaccagagcaggcgcagtctgtggtacaccagatcttggacctcttgtggctcttcatggaggactatgaggtacaggattgcctgaagcagttgatgatgtcacttctacgtctctaccgattctcgcctattgtcccagacctgggtctacagatccactacctgcgcctcactatgtccatcctgagacacgagaagtcccgcaagttcctgcttagcaatgtcctttttgacatgctccggtccgtggtcttcttttatattaagagtcccctgcgtgtggaggaagctggcctgaaggaactcattcccaccacctggtggccccatcgctccagcagggagagcagagacggtaaggaagcaagggaggagaccaccgaagagcggcagcggaggcgagcctatgagcgtggctgccaaagactcaagaaacgcattgaagtggtggaagaactgcaggtccagatcctgaagctgctgttggacaataaagatgacaatgggggtgaagcttctaggtacatctttctgacaaaattccgaaagttcctgcaggagaatgccagcggccgggggaacacacccgtgctctgcccccctgagtacatggtctgcttcctacaccggctggtgtctgccttgcgcttctattgggatgaatacaaagcttccaacccccgtgcttccttcagtgaggaggcttacatcccgccccagatcttctataatggcaaggtggactactttgaccttcagcgccttgggggcctcctctcacaccttcgaaagacccttaaagatgaccttgcttccaaagccaacatcgtgatcgaccccctggagctccaggcagccaccatggatgacctggatgaggatgaagagcctgccccctcagcggcccagcgtccgatgcaagccctggccatcggaggggcactgcccctgccccggccaggctggctcagttctccaaccctgggcagagccaaccgcttcctcagcacggcagctgtgagcctcatgaccccacggcggcttctgagcaccatggagaaagtcaaagttcgctcactgaatgtggaacagaggacccgtgaggacattgagggcagccactggaatgagggcctgctgttggggaggccccctgaagagcctgagcagccgcttaccgagaactcgctgttggaagtcctggatggcacagtcatgatgtataacctcagcgttcaccagcagctgggcaagatggtgggtgtgtctgatgatgtcaacgagtatgcaatggccctaagagacacagaggacaagctccgtcggtgccctaagaggaggaaggatatccttgcagagttgaccaagagccagaaggttttctcagaaaagctggaccacctgagccgcaggcttgcctgggtccacgccacagtctactcacaggagaaaatgctggatatctactggttactgcgtgtctgcctacggaccattgagcatggggaccgcacggggtctctctttgccttcatgcctgagttctacctaagtgtggctatcaacagctacagtgccctgaagaactattttggccctgtgcacagcatggaggaactcccaggctatgaagagaccctgacacgcttagctgccatcctcgccaaacactttgctgaccctcgaatagtaggcactgatattcgagactcactgatgcaggccctggccagctatgtgtgctacccacactccctgcgggctgtggaacggattcctgaggaacagcgcatcgccatggtgaggaaccttttggcaccctatgagcaacggccctgggcccagaccaactggatcctggtgcggctttggaggggctgtgggtttgggtaccgctatacacggctgccacatctgctgaaaaccaagccagaggatgccaatttgcccagcctccaaaagccctgcccttcgaccttgctacagcagcacatggcggacctgctgcgacaagggtctgatgtggcaccgagcttcctcaacagtgtccttaaccagctcaactgggccttctctgagttcatcggcatgatccaggagattcaacaggctgctgaacgcctggagcggaactttgtggacagccgacagctcaaggtctgtgccacctgctttgacctgtcggtcagcttgttgcgcgtcttggaaatgaccatcacgctggtacctgaaatattccttgactggtcccgccctacctctgagatgctgcttcggcgtctggcacagctgctgaaccaggtgctgaaccgggtgacagctgagaggaacctgtttgaccgtgtagttaccctacggctacctgggctggagagtgtggaccactaccctatcctggtggcagtgactggcatcctggtacgcctcctggtgcacggcccaacctcagagacagagcaagccacctctgtgctcctggctgatccctgcttccagcttcgttccatatgctatctcctggggcagccagagcccctagcacctggcactaccttgcctgcccctgaccggaaacgcttctctctacagagttatacagattatatcagcgctgaggagctggcccaggtggaacagatgctggctcacctgaccgctgcatctgcccaggcggccgccgcctccctgcccaccaatgaagaggacctctgcccaatctgctacgcccaccccatctctgctgtgttccagccttgtggtcacaaatcctgcaaagcctgcatcaaccagcacctgatgaacaacaaggactgcttcttctgcaaagccaccattgtatctgtagaggactgggacaaggcagccaacacaagcgccatgtcctcagctgcctag

SEQ ID NO: 8 - DNA, 41 bp, Artificial Sequence
  Artificial sequance
ccagaacatttggaccagttggctacaggtggacaatgagg

SEQ ID NO: 9 - DNA, 41 bp, Artificial Sequence
  Artificial sequance
gtgctgagtgatgccaggacacatcctggaagagaacatcc

SEQ ID NO: 10 - protein, 26 aa, Artificial Sequence
  Artificial sequance
  MISC_FEATURE (12)..(12): Serine (S) can be altered by Proline (P)
  MISC_FEATURE (17)..(17): Serine (S) can be altered by Proline (P)
  MISC_FEATURE (17)..(17): The Serine (S) may be phosphorylated
DELRDSDSVCDSGVETSFRKLSFTES

SEQ ID NO: 11 - RNA, 19 nt, Artificial Sequence
  Artificial sequnnce
gcgcuacuauugggaugaa

SEQ ID NO: 12 - RNA, 19 nt, Artificial Sequence
  Artificial sequance
caacugggccuucucugaa

SEQ ID NO: 13 - RNA, 19 nt, Artificial Sequence
  Artificial sequance
gcacauggcggaccuccua

SEQ ID NO: 14 - RNA, 19 nt, Artificial Sequence
  Artificial sequance
ggugaagcuucuagguaua

SEQ ID NO: 15 - RNA, 19 nt, Artificial Sequence
  Artificial sequance
gcuaauugaacacgcagaa

SEQ ID NO: 16 - RNA, 19 nt, Artificial Sequence
  Artificial sequance
gcacguagguggcguuguu

SEQ ID NO: 17 - RNA, 19 nt, Artificial Sequence
  Artificial sequance
cagaaugccgcgugcgagu

SEQ ID NO: 18 - RNA, 19 nt, Artificial Sequence
  Artificial sequance
agagaugagcugacggaaa